European Patent Specification EP 3 805 396 B1, published September 11, 2024. Title: Novel vectors and use thereof. Applicant: NATIONAL UNIVERSITY CORPORATION HOKKAIDO UNIVERSITY Fuso Pharmaceutical Industries, Ltd. The sequence listing filed with the application follows.

SEQUENCE LISTING (19 sequences)

SEQ ID NO: 1 - DNA, 1551 bp, Homo sapiens
ggccctccgcgcctacagctcaagccacatccgaagggggagggagccgggagctgcgcgcggggccgccggggggaggggtggcaccgcccacgccgggcggccacgaagggcggggcagcgggcgcgcgcgcggcggggggaggggccggcgccgcgcccgctgggaattggggccctagggggagggcggaggcgccgacgaccgcggcacttaccgttcgcggcgtggcgcccggtggtccccaaggggagggaagggggaggcggggcgaggacagtgaccggagtctcctcagcggtggcttttctgcttggcagcctcagcggctggcgccaaaaccggactccgcccacttcctcgcccgccggtgcgagggtgtggaatcctccagacgctgggggagggggagttgggagcttaaaaactagtacccctttgggaccactttcagcagcgaactctcctgtacaccaggggtcagttccacagacgcgggccaggggtgggtcattgcggcgtgaacaataatttgactagaagttgattcgggtgtttccggaaggggccgagtcaatccgccgagttggggcacggaaaacaaaaagggaaggctactaagatttttctggcgggggttatcattggcgtaactgcagggaccacctcccgggttgagggggctggatctccaggctgcggattaagcccctcccgtcggcgttaatttcaaactgcgcgacgtttctcacctgccttcgccaaggcaggggccgggaccctattccaagaggtagtaactagcaggactctagccttccgcaattcattgagcgcatttacggaagtaacgtcgggtactgtctctggccgcaagggtgggaggagtacgcatttggcgtaaggtggggcgtagagccttcccgccattggcggcggatagggcgtttacgcgacggcctgacgtagcggaagacgccttagtgggggggaaggttctagaaaagcggcggcagcggctctagcggcagtagcagcagcgccgggtcccgtgcggaggtgctcctcgcagagttgtttctccagcagcggcagttctcactacagcgccaggacgagtccggttcgtgttcgtccgcggagatctctctcatctcgctcggctgcgggaaatcgggctgaagcgactgagtccgcgatggaggtaacgggtttgaaatcaatgagttattgaaaagggcatggcgaggccgttggcgcctcagtggaagtcggccagccgcctccgtgggagagaggcaggaaatcggaccaattcagtagcagtggggcttaaggtttatgaacggggtcttgagcggaggcctgagcgtacaaacagcttccccaccctcagcctcccggcgccatttcccttcactgggggtgggggatggggagctttcacatggcggacgctgccccgctggggtgaaagtggggcgcggaggcgggacttcttattccctttctaaagcacgctgcttcgggggccacggcgtctcctcgga

SEQ ID NO: 2 - DNA, 15 bp, Artificial Sequence
  Optimized Kozak sequence
ccgccgccaccatgg

SEQ ID NO: 3 - DNA, 11327 bp, Artificial Sequence
  pDC62c5-U533
cgatgtacgggccagatatacgcgttgacattgattattgactagtcgcgttacataacttacggtaaatggcccgcctggctgaccgcccaacgacccccgcccattgacgtcaataatgacgtatgttcccatagtaacgccaatagggactttccattgacgtcaatgggtggagtatttacggtaaactgcccacttggcagtacatcaagtgtatcatatgccaagtccgccccctattgacgtcaatgacggtaaatggcccgcctggcattatgcccagtacatgaccttacgggactttcctacttggcagtacatctacgtattagtcatcgctattaccatggtgatgcggttttggcagtacaccaatgggcgtggatagcggtttgactcacggggatttccaagtctccaccccattgacgtcaatgggagtttgttttggcaccaaaatcaacgggactttccaaaatgtcgtaataaccccgccccgttgacgcaaatgggcggtaggcgtgtacggtgggaggtctatataagcagagctcgtttagtgaaccgtcagatcctcactctcttccgcatcgctgtctgcgagggccagctgttgggctcgcggttgaggacaaactcttcgcggtctttccagtactcttggatcggaaacccgtcggcctccgaacggtactccgccaccgagggacctgagcgagtccgcatcgaccggatcggaaaacctctcgagaaaggcgtctaaccagtcacagtcgcaaggtaggctgagcaccgtggcgggcggcagcgggtggcggtcggggttgtttctggcggaggtgctgctgatgatgtaattaaagtaggcggtcttgagacggcggatggtcgaggtgaggtgtggcaggcttgagatccagctgttggggtgagtactccctctcaaaagcgggcatgacttctgcgctaagattgtcagtttccaaaaacgaggaggatttgatattcacctggcccgatctggccatacacttgagtgacaatgacatccactttgcctttctctccacaggtgtccactcccaggtccaaggcgcgccgcgatcgcgcctcgactgtgccttctagttgccagccatctgttgtttgcccctcccccgtgccttccttgaccctggaaggtgccactcccactgtcctttcctaataaaatgaggaaattgcatcgcattgtctgagtaggtgtcattctattctggggggtggggtggggcaggacagcaagggggaggattgggaagacaatagcaggcatgctggggaggatctccgcggggccctccgcgcctacagctcaagccacatccgaagggggagggagccgggagctgcgcgcggggccgccggggggaggggtggcaccgcccacgccgggcggccacgaagggcggggcagcgggcgcgcgcgcggcggggggaggggccggcgccgcgcccgctgggaattggggccctagggggagggcggaggcgccgacgaccgcggcacttaccgttcgcggcgtggcgcccggtggtccccaaggggagggaagggggaggcggggcgaggacagtgaccggagtctcctcagcggtggcttttctgcttggcagcctcagcggctggcgccaaaaccggactccgcccacttcctcgcccgccggtgcgagggtgtggaatcctccagacgctgggggagggggagttgggagcttaaaaactagtacccctttgggaccactttcagcagcgaactctcctgtacaccaggggtcagttccacagacgcgggccaggggtgggtcattgcggcgtgaacaataatttgactagaagttgattcgggtgtttccggaaggggccgagtcaatccgccgagttggggcacggaaaacaaaaagggaaggctactaagatttttctggcgggggttatcattggcgtaactgcagggaccacctcccgggttgagggggctggatctccaggctgcggattaagcccctcccgtcggcgttaatttcaaactgcgcgacgtttctcacctgccttcgccaaggcaggggccgggaccctattccaagaggtagtaactagcaggactctagccttccgcaattcattgagcgcatttacggaagtaacgtcgggtactgtctctggccgcaagggtgggaggagtacgcatttggcgtaaggtggggcgtagagccttcccgccattggcggcggatagggcgtttacgcgacggcctgacgtagcggaagacgccttagtgggggggaaggttctagaaaagcggcggcagcggctctagcggcagtagcagcagcgccgggtcccgtgcggaggtgctcctcgcagagttgtttctccagcagcggcagttctcactacagcgccaggacgagtccggttcgtgttcgtccgcggagatctctctcatctcgctcggctgcgggaaatcgggctgaagcgactgagtccgcgatggaggtaacgggtttgaaatcaatgagttattgaaaagggcatggcgaggccgttggcgcctcagtggaagtcggccagccgcctccgtgggagagaggcaggaaatcggaccaattcagtagcagtggggcttaaggtttatgaacggggtcttgagcggaggcctgagcgtacaaacagcttccccaccctcagcctcccggcgccatttcccttcactgggggtgggggatggggagctttcacatggcggacgctgccccgctggggtgaaagtggggcgcggaggcgggacttcttattccctttctaaagcacgctgcttcgggggccacggcgtctcctcggagaattccgatgtacgggccagatatacgcgttgacattgattattgactagtcgcgttacataacttacggtaaatggcccgcctggctgaccgcccaacgacccccgcccattgacgtcaataatgacgtatgttcccatagtaacgccaatagggactttccattgacgtcaatgggtggagtatttacggtaaactgcccacttggcagtacatcaagtgtatcatatgccaagtccgccccctattgacgtcaatgacggtaaatggcccgcctggcattatgcccagtacatgaccttacgggactttcctacttggcagtacatctacgtattagtcatcgctattaccatggtgatgcggttttggcagtacaccaatgggcgtggatagcggtttgactcacggggatttccaagtctccaccccattgacgtcaatgggagtttgttttggcaccaaaatcaacgggactttccaaaatgtcgtaataaccccgccccgttgacgcaaatgggcggtaggcgtgtacggtgggaggtctatataagcagagctcgtttagtgaaccgtcagatcctcactctcttccgcatcgctgtctgcgagggccagctgttgggctcgcggttgaggacaaactcttcgcggtctttccagtactcttggatcggaaacccgtcggcctccgaacggtactccgccaccgagggacctgagcgagtccgcatcgaccggatcggaaaacctctcgagaaaggcgtctaaccagtcacagtcgcaaggtaggctgagcaccgtggcgggcggcagcgggtggcggtcggggttgtttctggcggaggtgctgctgatgatgtaattaaagtaggcggtcttgagacggcggatggtcgaggtgaggtgtggcaggcttgagatccagctgttggggtgagtactccctctcaaaagcgggcatgacttctgcgctaagattgtcagtttccaaaaacgaggaggatttgatattcacctggcccgatctggccatacacttgagtgacaatgacatccactttgcctttctctccacaggtgtccactcccaggtccaagcggccgccctgcagggcctcgactgtgccttctagttgccagccatctgttgtttgcccctcccccgtgccttccttgaccctggaaggtgccactcccactgtcctttcctaataaaatgaggaaattgcatcgcattgtctgagtaggtgtcattctattctggggggtggggtggggcaggacagcaagggggaggattgggaagacaatagcaggcatgctggggaggatctccgcggggccctccgcgcctacagctcaagccacatccgaagggggagggagccgggagctgcgcgcggggccgccggggggaggggtggcaccgcccacgccgggcggccacgaagggcggggcagcgggcgcgcgcgcggcggggggaggggccggcgccgcgcccgctgggaattggggccctagggggagggcggaggcgccgacgaccgcggcacttaccgttcgcggcgtggcgcccggtggtccccaaggggagggaagggggaggcggggcgaggacagtgaccggagtctcctcagcggtggcttttctgcttggcagcctcagcggctggcgccaaaaccggactccgcccacttcctcgcccgccggtgcgagggtgtggaatcctccagacgctgggggagggggagttgggagcttaaaaactagtacccctttgggaccactttcagcagcgaactctcctgtacaccaggggtcagttccacagacgcgggccaggggtgggtcattgcggcgtgaacaataatttgactagaagttgattcgggtgtttccggaaggggccgagtcaatccgccgagttggggcacggaaaacaaaaagggaaggctactaagatttttctggcgggggttatcattggcgtaactgcagggaccacctcccgggttgagggggctggatctccaggctgcggattaagcccctcccgtcggcgttaatttcaaactgcgcgacgtttctcacctgccttcgccaaggcaggggccgggaccctattccaagaggtagtaactagcaggactctagccttccgcaattcattgagcgcatttacggaagtaacgtcgggtactgtctctggccgcaagggtgggaggagtacgcatttggcgtaaggtggggcgtagagccttcccgccattggcggcggatagggcgtttacgcgacggcctgacgtagcggaagacgccttagtgggggggaaggttctagaaaagcggcggcagcggctctagcggcagtagcagcagcgccgggtcccgtgcggaggtgctcctcgcagagttgtttctccagcagcggcagttctcactacagcgccaggacgagtccggttcgtgttcgtccgcggagatctctctcatctcgctcggctgcgggaaatcgggctgaagcgactgagtccgcgatggaggtaacgggtttgaaatcaatgagttattgaaaagggcatggcgaggccgttggcgcctcagtggaagtcggccagccgcctccgtgggagagaggcaggaaatcggaccaattcagtagcagtggggcttaaggtttatgaacggggtcttgagcggaggcctgagcgtacaaacagcttccccaccctcagcctcccggcgccatttcccttcactgggggtgggggatggggagctttcacatggcggacgctgccccgctggggtgaaagtggggcgcggaggcgggacttcttattccctttctaaagcacgctgcttcgggggccacggcgtctcctcggaaccggttgtggaatgtgtgtcagttagggtgtggaaagtccccaggctccccagcaggcagaagtatgcaaagcatgcatctcaattagtcagcaaccatagtcccgcccctaactccgcccatcccgcccctaactccgcccagttccgcccattctccgccccatggctgactaattttttttatttatgcagaggccgaggccgcctcggcctctgagctattccagaagtagtgaggaggcttttttggaggcctaggcttttgcaaaaaagctgcagatggtacgaccattaaattgtattgtagcagtatcacaaaatatgggtattggtaaaaatggtgatttaccatggccaccattacgaaatgaatttaaatattttcaacgaatgactactacttcatcagtagaaggtaaacaaaatttagtaattatgggtcgaaaaacttggttttcaattcctgagaagaatcgacctttaaaggacagaattaatatagttctcagtagagaactcaaagaaccaccacgaggagctcattttcttgccaaaagtttggatgatgccttaagacttattgaacaaccggaattggcaagtaaagtagacatggtttggatagtcggaggcagttctgtttaccaggaagccatgaatcaaccaggccacctcagactctttgtgacaaggatcatgcaggaatttgaaagtgacacgtttttcccagaaattgatttggggaaatataaacttctcccagaatacccaggcgtcctctctgaggtccaggaggaaaaaggcatcaagtataagtttgaagtctacgagaagaaagactaaagatccgtgacataattggacaaactacctacagagatttaaagctctaaggtaaatataaaatttttaagtgtataatgtgttaaactactgattctaattgtttgtgtattttagattccaacctatggaactgatgaatgggagcagtggtggaatgcctttaatgaggaaaacctgttttgctcagaagaaatgccatctagtgatgatgaggctactgctgactctcaacattctactcctccaaaaaagaagagaaaggtagaagaccccaaggactttccttcagaattgctaagttttttgagtcatgctgtgtttagtaatagaactcttgcttgctttgctatttacaccacaaaggaaaaagctgcactgctatacaagaaaattatggaaaaatattctgtaacctttataagtaggcataacagttataatcataacatactgttttttcttactccacacaggcatagagtgtctgctattaataactatgctcaaaaattgtgtacctttagctttttaatttgtaaaggggttaataaggaatatttgatgtatagtgccttgactagagatcataatcagccataccacatttgtagaggttttacttgctttaaaaaacctcccacacctccccctgaacctgaaacataaaatgaatgcaattgttgttgttaacttgtttattgcagcttataatggttacaaataaagcaatagcatcacaaatttcacaaataaagcatttttttcactgcattctagttgtggtttgtccaaactcatcaatgtatcttatcatgtctgggcccatcgatgccgacgtagcgcctgatgcggtattttctccttacgcatctgtgcggtatttcacaccgcatatggtgcactctcagtacaatctgctctgatgccgcatagttaagccagccccgacacccgccaacacccgctgacgcgccctgacgggcttgtctgctcccggcatccgcttacagacaagctgtgaccgtctccgggagctgcatgtgtcagaggttttcaccgtcatcaccgaaacgcgcgagacgaaagggcctcgtgatacgcctatttttataggttaatgtcatgataataatggtttcttagacgtcaggtggcacttttcggggaaatgtgcgcggaacccctatttgtttatttttctaaatacattcaaatatgtatccgctcatgagacaataaccctgataaatgcttcaataatattgaaaaaggaagagtatgagtattcaacatttccgtgtcgcccttattcccttttttgcggcattttgccttcctgtttttgctcacccagaaacgctggtgaaagtaaaagatgctgaagatcagttgggtgcacgagtgggttacatcgaactggatctcaacagcggtaagatccttgagagttttcgccccgaagaacgttttccaatgatgagcacttttaaagttctgctatgtggcgcggtattatcccgtattgacgccgggcaagagcaactcggtcgccgcatacactattctcagaatgacttggttgagtactcaccagtcacagaaaagcatcttacggatggcatgacagtaagagaattatgcagtgctgccataaccatgagtgataacactgcggccaacttacttctgacaacgatcggaggaccgaaggagctaaccgcttttttgcacaacatgggggatcatgtaactcgccttgatcgttgggaaccggagctgaatgaagccataccaaacgacgagcgtgacaccacgatgcctgtagcaatggcaacaacgttgcgcaaactattaactggcgaactacttactctagcttcccggcaacaattaatagactggatggaggcggataaagttgcaggaccacttctgcgctcggcccttccggctggctggtttattgctgataaatctggagccggtgagcgtgggtctcgcggtatcattgcagcactggggccagatggtaagccctcccgtatcgtagttatctacacgacggggagtcaggcaactatggatgaacgaaatagacagatcgctgagataggtgcctcactgattaagcattggtaactgtcagaccaagtttactcatatatactttagattgatttaaaacttcatttttaatttaaaaggatctaggtgaagatcctttttgataatctcatgaccaaaatcccttaacgtgagttttcgttccactgagcgtcagaccccgtagaaaagatcaaaggatcttcttgagatcctttttttctgcgcgtaatctgctgcttgcaaacaaaaaaaccaccgctaccagcggtggtttgtttgccggatcaagagctaccaactctttttccgaaggtaactggcttcagcagagcgcagataccaaatactgttcttctagtgtagccgtagttaggccaccacttcaagaactctgtagcaccgcctacatacctcgctctgctaatcctgttaccagtggctgctgccagtggcgataagtcgtgtcttaccgggttggactcaagacgatagttaccggataaggcgcagcggtcgggctgaacggggggttcgtgcacacagcccagcttggagcgaacgacctacaccgaactgagatacctacagcgtgagctatgagaaagcgccacgcttcccgaagggagaaaggcggacaggtatccggtaagcggcagggtcggaacaggagagcgcacgagggagcttccagggggaaacgcctggtatctttatagtcctgtcgggtttcgccacctctgacttgagcgtcgatttttgtgatgctcgtcaggggggcggagcctatggaaaaacgccagcaacgcggcctttttacggttcctggccttttgctggccttttgctcacatgttctttcctgcgttatcccctgattctgtggataaccgtattaccgcctttgagtgagctgataccgctcgccgcagccgaacgaccgagcgcagcgagtcagtgagcgaggaagcggaagagcgcccaatacgcaaaccgcctctccccgcgcgttggccgattcattaatgcagctgggccctccgcgcctacagctcaagccacatccgaagggggagggagccgggagctgcgcgcggggccgccggggggaggggtggcaccgcccacgccgggcggccacgaagggcggggcagcgggcgcgcgcgcggcggggggaggggccggcgccgcgcccgctgggaattggggccctagggggagggcggaggcgccgacgaccgcggcacttaccgttcgcggcgtggcgcccggtggtccccaaggggagggaagggggaggcggggcgaggacagtgaccggagtctcctcagcggtggcttttctgcttggcagcctcagcggctggcgccaaaaccggactccgcccacttcctcgcccgccggtgcgagggtgtggaatcctccagacgctgggggagggggagttgggagcttaaaaactagtacccctttgggaccactttcagcagcgaactctcctgtacaccaggggtcagttccacagacgcgggccaggggtgggtcattgcggcgtgaacaataatttgactagaagttgattcgggtgtttccggaaggggccgagtcaatccgccgagttggggcacggaaaacaaaaagggaaggctactaagatttttctggcgggggttatcattggcgtaactgcagggaccacctcccgggttgagggggctggatctccaggctgcggattaagcccctcccgtcggcgttaatttcaaactgcgcgacgtttctcacctgccttcgccaaggcaggggccgggaccctattccaagaggtagtaactagcaggactctagccttccgcaattcattgagcgcatttacggaagtaacgtcgggtactgtctctggccgcaagggtgggaggagtacgcatttggcgtaaggtggggcgtagagccttcccgccattggcggcggatagggcgtttacgcgacggcctgacgtagcggaagacgccttagtgggggggaaggttctagaaaagcggcggcagcggctctagcggcagtagcagcagcgccgggtcccgtgcggaggtgctcctcgcagagttgtttctccagcagcggcagttctcactacagcgccaggacgagtccggttcgtgttcgtccgcggagatctctctcatctcgctcggctgcgggaaatcgggctgaagcgactgagtccgcgatggaggtaacgggtttgaaatcaatgagttattgaaaagggcatggcgaggccgttggcgcctcagtggaagtcggccagccgcctccgtgggagagaggcaggaaatcggaccaattcagtagcagtggggcttaaggtttatgaacggggtcttgagcggaggcctgagcgtacaaacagcttccccaccctcagcctcccggcgccatttcccttcactgggggtgggggatggggagctttcacatggcggacgctgccccgctggggtgaaagtggggcgcggaggcgggacttcttattccctttctaaagcacgctgcttcgggggccacggcgtctcctcggaaagctt

SEQ ID NO: 4 - DNA, 736 bp, Artificial Sequence
  Antibody (OMLH) light chain gene cDNA with optimized Kozak sequence added upstream of the initiation codon
cgcgccccgccgccaccatgggttggtcttgtatcatcttatttttagttgctactgctactggtgttcattctgatatacagctcacccaaagcccatcatctctgtctgcaagcgtcggcgacagggtgaccattacctgtcgcgcaagccaaagcgttgactacgacggcgacagctacatgaactggtaccagcagaagcccggcaaggctcctaagctgctgatctatgccgcctcctaccttgaatctggagtgccttctcgtttttccggctcagggtccggaactgattttaccctgaccatttcctccctccagcccgaggattttgccacttactactgtcagcagtcccacgaggacccatatacattcggacaaggtacaaaggtagaaatcaagcgtacggtggctgccccatccgtgttcatatttcctcctagcgacgaacaactcaagtccggtaccgccagcgtggtctgcctgttgaacaatttttatccaagagaagctaaggtccagtggaaggttgacaacgcccttcagtccggaaatagccaagagagcgtcaccgaacaggactccaaggacagtacatactcactgagctctacactgaccctttctaaggccgactacgagaagcacaaggtctacgcatgcgaagtgacccatcagggactcagtagccctgtaacaaagagttttaatcgaggcgagtgctaagcgat

SEQ ID NO: 5 - DNA, 1436 bp, Artificial Sequence
  Antibody (OMLH) heavy chain gene cDNA with optimized Kozak sequence added upstream of the initiation codon
ggccgcccgccgccaccatggaatttggtttatcttgggtttttttagttgctttattaagaggtgttcaatgtgaggtgcagttggtcgaatccggcggcggactcgtgcaaccaggcggaagtttgcggctgtcctgcgcagtgtctggttacagcatcacctccgggtatagctggaactggatccgccaggctcctggaaaggggcttgagtgggtggcttccattacctacgacggctccactaactataacccgagcgtcaaaggcagaatcaccatctctcgggacgactcaaagaataccttctacctgcagatgaactcactgagggccgaagataccgcagtttactactgcgccagggggtcccactatttcggccactggcacttcgccgtgtggggacagggcacactcgtgaccgttagtagcgctagcaccaaaggcccctctgtgttcccacttgctccctccagtaaatctacctccggaggaaccgcagccctcggctgcctggtgaaggattacttcccagagcccgtcaccgtctcttggaactccggagccttgactagcggagtgcacactttccctgctgtattgcagtccagcggcttgtattcactgagtagcgtcgtcaccgtgccttcaagcagcctcgggacacagacatacatatgtaatgtcaaccataagccatcaaacactaaagttgataaaaaggtggaacctaagagttgcgataagacccatacctgtcctccttgccctgctcctgagctgctgggaggccctagcgtgtttctgttcccccccaagcccaaagatacactgatgatttcccgcacacctgaagtaacatgtgtcgtggttgatgtgagtcacgaggatccagaggtcaagtttaattggtacgtggacggagtggaggtgcacaacgctaagactaagcctcgggaggaacagtacaacagcacataccgcgtggtcagcgttttgactgtgctgcatcaagactggctcaatggaaaggaatacaagtgcaaggtctctaataaagccctccccgctcctattgagaagactatttctaaagccaagggccagcctcgcgaacctcaggtatatactttgccaccctctcgcgaagaaatgacaaagaatcaggtctcactcacttgcctcgtcaaagggttttacccttctgacatcgctgtcgaatgggaaagtaatggtcagccagaaaacaattacaagactactccaccagtgctcgattctgatggaagtttctttctctacagtaagctcactgtggacaaatctcgctggcagcagggtaacgtattctcatgctccgtgatgcatgaagccctccacaaccattacacccagaagagcctgtctctgagcccaggcaagtaacctgca

SEQ ID NO: 6 - DNA, 7317 bp, Artificial Sequence
  pDC61
cgatgtacgggccagatatacgcgttgacattgattattgactagttattaatagtaatcaattacggggtcattagttcatagcccatatatggagttccgcgttacataacttacggtaaatggcccgcctggctgaccgcccaacgacccccgcccattgacgtcaataatgacgtatgttcccatagtaacgccaatagggactttccattgacgtcaatgggtggagtatttacggtaaactgcccacttggcagtacatcaagtgtatcatatgccaagtacgccccctattgacgtcaatgacggtaaatggcccgcctggcattatgcccagtacatgaccttatgggactttcctacttggcagtacatctacgtattagtcatcgctattaccatggtgatgcggttttggcagtacatcaatgggcgtggatagcggtttgactcacggggatttccaagtctccaccccattgacgtcaatgggagtttgttttggcaccaaaatcaacgggactttccaaaatgtcgtaacaactccgccccattgacgcaaatgggcggtaggcgtgtacggtgggaggtctatataagcagagctctctggctaactagagaacccactgttaactggcttatcgaaattgtcgaggagaacttcagggtgagtttggggacccttgattgttctttctttttcgctattgtaaaattcatgttatatggagggggcaaagttttcagggtgttgtttagaatgggaagatgtcccttgtatcaccatggaccctcatgataattttgtttctttcactttctactctgttgacaaccattgtctcctcttattttcttttcattttctgtaactttttcgttaaactttagcttgcatttgtaacgaatttttaaattcacttttgtttatttgtcagattgtaagtactttctctaatcacttttttttcaaggcaatcagggtatattatattgtacttcagcacagttttagagaacaattgttataattaaatgataaggtagaatatttctgcatataaattctggctggcgtggaaatattcttattggtagaaacaactacatcctggtcatcatcctgcctttctctttatggttacaatgatatacactgtttgagatgaggataaaatactctgagtccaaaccgggcccctctgctaaccatgttcatgccttcttctttttcctacagctcctgggcaacgtgctggcggccgccccggggcctcgactgtgccttctagttgccagccatctgttgtttgcccctcccccgtgccttccttgaccctggaaggtgccactcccactgtcctttcctaataaaatgaggaaattgcatcgcattgtctgagtaggtgtcattctattctggggggtggggtggggcaggacagcaagggggaggattgggaagacaatagcaggcatgctggggactcgagcgatgtacgggccagatatacgcgttgacattgattattgactagttattaatagtaatcaattacggggtcattagttcatagcccatatatggagttccgcgttacataacttacggtaaatggcccgcctggctgaccgcccaacgacccccgcccattgacgtcaataatgacgtatgttcccatagtaacgccaatagggactttccattgacgtcaatgggtggagtatttacggtaaactgcccacttggcagtacatcaagtgtatcatatgccaagtacgccccctattgacgtcaatgacggtaaatggcccgcctggcattatgcccagtacatgaccttatgggactttcctacttggcagtacatctacgtattagtcatcgctattaccatggtgatgcggttttggcagtacatcaatgggcgtggatagcggtttgactcacggggatttccaagtctccaccccattgacgtcaatgggagtttgttttggcaccaaaatcaacgggactttccaaaatgtcgtaacaactccgccccattgacgcaaatgggcggtaggcgtgtacggtgggaggtctatataagcagagctctctggctaactagagaacccactgttaactggcttatcgaaattgtcgaggagaacttcagggtgagtttggggacccttgattgttctttctttttcgctattgtaaaattcatgttatatggagggggcaaagttttcagggtgttgtttagaatgggaagatgtcccttgtatcaccatggaccctcatgataattttgtttctttcactttctactctgttgacaaccattgtctcctcttattttcttttcattttctgtaactttttcgttaaactttagcttgcatttgtaacgaatttttaaattcacttttgtttatttgtcagattgtaagtactttctctaatcacttttttttcaaggcaatcagggtatattatattgtacttcagcacagttttagagaacaattgttataattaaatgataaggtagaatatttctgcatataaattctggctggcgtggaaatattcttattggtagaaacaactacatcctggtcatcatcctgcctttctctttatggttacaatgatatacactgtttgagatgaggataaaatactctgagtccaaaccgggcccctctgctaaccatgttcatgccttcttctttttcctacagctcctgggcaacgtgctggcgcgcctctagagcctcgactgtgccttctagttgccagccatctgttgtttgcccctcccccgtgccttccttgaccctggaaggtgccactcccactgtcctttcctaataaaatgaggaaattgcatcgcattgtctgagtaggtgtcattctattctggggggtggggtggggcaggacagcaagggggaggattgggaagacaatagcaggcatgctggggaggatctccgcggtgtggaatgtgtgtcagttagggtgtggaaagtccccaggctccccagcaggcagaagtatgcaaagcatgcatctcaattagtcagcaaccatagtcccgcccctaactccgcccatcccgcccctaactccgcccagttccgcccattctccgccccatggctgactaattttttttatttatgcagaggccgaggccgcctcggcctctgagctattccagaagtagtgaggaggcttttttggaggcctaggcttttgcaaaaaagctgcagatggtacgaccattaaattgtattgtagcagtatcacaaaatatgggtattggtaaaaatggtgatttaccatggccaccattacgaaatgaatttaaatattttcaacgaatgactactacttcatcagtagaaggtaaacaaaatttagtaattatgggtcgaaaaacttggttttcaattcctgagaagaatcgacctttaaaggacagaattaatatagttctcagtagagaactcaaagaaccaccacgaggagctcattttcttgccaaaagtttggatgatgccttaagacttattgaacaaccggaattggcaagtaaagtagacatggtttggatagtcggaggcagttctgtttaccaggaagccatgaatcaaccaggccacctcagactctttgtgacaaggatcatgcaggaatttgaaagtgacacgtttttcccagaaattgatttggggaaatataaacttctcccagaatacccaggcgtcctctctgaggtccaggaggaaaaaggcatcaagtataagtttgaagtctacgagaagaaagactaaagatccgtgacataattggacaaactacctacagagatttaaagctctaaggtaaatataaaatttttaagtgtataatgtgttaaactactgattctaattgtttgtgtattttagattccaacctatggaactgatgaatgggagcagtggtggaatgcctttaatgaggaaaacctgttttgctcagaagaaatgccatctagtgatgatgaggctactgctgactctcaacattctactcctccaaaaaagaagagaaaggtagaagaccccaaggactttccttcagaattgctaagttttttgagtcatgctgtgtttagtaatagaactcttgcttgctttgctatttacaccacaaaggaaaaagctgcactgctatacaagaaaattatggaaaaatattctgtaacctttataagtaggcataacagttataatcataacatactgttttttcttactccacacaggcatagagtgtctgctattaataactatgctcaaaaattgtgtacctttagctttttaatttgtaaaggggttaataaggaatatttgatgtatagtgccttgactagagatcataatcagccataccacatttgtagaggttttacttgctttaaaaaacctcccacacctccccctgaacctgaaacataaaatgaatgcaattgttgttgttaacttgtttattgcagcttataatggttacaaataaagcaatagcatcacaaatttcacaaataaagcatttttttcactgcattctagttgtggtttgtccaaactcatcaatgtatcttatcatgtctgggcccatcgatgaattcactggccgtcgttttacaacgtcgtgactgggaaaaccctggcgttacccaacttaatcgccttgcagcacatccccctttcgccagctggcgtaatagcgaagaggcccgcaccgatcgcccttcccaacagttgcgcagcctgaatggcgaatggcgcctgatgcggtattttctccttacgcatctgtgcggtatttcacaccgcatatggtgcactctcagtacaatctgctctgatgccgcatagttaagccagccccgacacccgccaacacccgctgacgcgccctgacgggcttgtctgctcccggcatccgcttacagacaagctgtgaccgtctccgggagctgcatgtgtcagaggttttcaccgtcatcaccgaaacgcgcgagacgaaagggcctcgtgatacgcctatttttataggttaatgtcatgataataatggtttcttagacgtcaggtggcacttttcggggaaatgtgcgcggaacccctatttgtttatttttctaaatacattcaaatatgtatccgctcatgagacaataaccctgataaatgcttcaataatattgaaaaaggaagagtatgagtattcaacatttccgtgtcgcccttattcccttttttgcggcattttgccttcctgtttttgctcacccagaaacgctggtgaaagtaaaagatgctgaagatcagttgggtgcacgagtgggttacatcgaactggatctcaacagcggtaagatccttgagagttttcgccccgaagaacgttttccaatgatgagcacttttaaagttctgctatgtggcgcggtattatcccgtattgacgccgggcaagagcaactcggtcgccgcatacactattctcagaatgacttggttgagtactcaccagtcacagaaaagcatcttacggatggcatgacagtaagagaattatgcagtgctgccataaccatgagtgataacactgcggccaacttacttctgacaacgatcggaggaccgaaggagctaaccgcttttttgcacaacatgggggatcatgtaactcgccttgatcgttgggaaccggagctgaatgaagccataccaaacgacgagcgtgacaccacgatgcctgtagcaatggcaacaacgttgcgcaaactattaactggcgaactacttactctagcttcccggcaacaattaatagactggatggaggcggataaagttgcaggaccacttctgcgctcggcccttccggctggctggtttattgctgataaatctggagccggtgagcgtgggtctcgcggtatcattgcagcactggggccagatggtaagccctcccgtatcgtagttatctacacgacggggagtcaggcaactatggatgaacgaaatagacagatcgctgagataggtgcctcactgattaagcattggtaactgtcagaccaagtttactcatatatactttagattgatttaaaacttcatttttaatttaaaaggatctaggtgaagatcctttttgataatctcatgaccaaaatcccttaacgtgagttttcgttccactgagcgtcagaccccgtagaaaagatcaaaggatcttcttgagatcctttttttctgcgcgtaatctgctgcttgcaaacaaaaaaaccaccgctaccagcggtggtttgtttgccggatcaagagctaccaactctttttccgaaggtaactggcttcagcagagcgcagataccaaatactgttcttctagtgtagccgtagttaggccaccacttcaagaactctgtagcaccgcctacatacctcgctctgctaatcctgttaccagtggctgctgccagtggcgataagtcgtgtcttaccgggttggactcaagacgatagttaccggataaggcgcagcggtcgggctgaacggggggttcgtgcacacagcccagcttggagcgaacgacctacaccgaactgagatacctacagcgtgagctatgagaaagcgccacgcttcccgaagggagaaaggcggacaggtatccggtaagcggcagggtcggaacaggagagcgcacgagggagcttccagggggaaacgcctggtatctttatagtcctgtcgggtttcgccacctctgacttgagcgtcgatttttgtgatgctcgtcaggggggcggagcctatggaaaaacgccagcaacgcggcctttttacggttcctggccttttgctggccttttgctcacatgttctttcctgcgttatcccctgattctgtggataaccgtattaccgcctttgagtgagctgataccgctcgccgcagccgaacgaccgagcgcagcgagtcagtgagcgaggaagcggaagagcgcccaatacgcaaaccgcctctccccgcgcgttggccgattcattaatgcagctggcacgacaggtttcccgactggaaagcgggcagtgagcgcaacgcaattaatgtgagttagctcactcattaggcaccccaggctttacactttatgcttccggctcgtatgttgtgtggaattgtgagcggataacaatttcacacaggaaacagctatgaccatgattacgccaagctt

SEQ ID NO: 7 - DNA, 2635 bp, Artificial Sequence
  Sequence in pDC61, which is substitued for the sequence from No. 3182 to No. 5843 in pDC6
aattcactggccgtcgttttacaacgtcgtgactgggaaaaccctggcgttacccaacttaatcgccttgcagcacatccccctttcgccagctggcgtaatagcgaagaggcccgcaccgatcgcccttcccaacagttgcgcagcctgaatggcgaatggcgcctgatgcggtattttctccttacgcatctgtgcggtatttcacaccgcatatggtgcactctcagtacaatctgctctgatgccgcatagttaagccagccccgacacccgccaacacccgctgacgcgccctgacgggcttgtctgctcccggcatccgcttacagacaagctgtgaccgtctccgggagctgcatgtgtcagaggttttcaccgtcatcaccgaaacgcgcgagacgaaagggcctcgtgatacgcctatttttataggttaatgtcatgataataatggtttcttagacgtcaggtggcacttttcggggaaatgtgcgcggaacccctatttgtttatttttctaaatacattcaaatatgtatccgctcatgagacaataaccctgataaatgcttcaataatattgaaaaaggaagagtatgagtattcaacatttccgtgtcgcccttattcccttttttgcggcattttgccttcctgtttttgctcacccagaaacgctggtgaaagtaaaagatgctgaagatcagttgggtgcacgagtgggttacatcgaactggatctcaacagcggtaagatccttgagagttttcgccccgaagaacgttttccaatgatgagcacttttaaagttctgctatgtggcgcggtattatcccgtattgacgccgggcaagagcaactcggtcgccgcatacactattctcagaatgacttggttgagtactcaccagtcacagaaaagcatcttacggatggcatgacagtaagagaattatgcagtgctgccataaccatgagtgataacactgcggccaacttacttctgacaacgatcggaggaccgaaggagctaaccgcttttttgcacaacatgggggatcatgtaactcgccttgatcgttgggaaccggagctgaatgaagccataccaaacgacgagcgtgacaccacgatgcctgtagcaatggcaacaacgttgcgcaaactattaactggcgaactacttactctagcttcccggcaacaattaatagactggatggaggcggataaagttgcaggaccacttctgcgctcggcccttccggctggctggtttattgctgataaatctggagccggtgagcgtgggtctcgcggtatcattgcagcactggggccagatggtaagccctcccgtatcgtagttatctacacgacggggagtcaggcaactatggatgaacgaaatagacagatcgctgagataggtgcctcactgattaagcattggtaactgtcagaccaagtttactcatatatactttagattgatttaaaacttcatttttaatttaaaaggatctaggtgaagatcctttttgataatctcatgaccaaaatcccttaacgtgagttttcgttccactgagcgtcagaccccgtagaaaagatcaaaggatcttcttgagatcctttttttctgcgcgtaatctgctgcttgcaaacaaaaaaaccaccgctaccagcggtggtttgtttgccggatcaagagctaccaactctttttccgaaggtaactggcttcagcagagcgcagataccaaatactgttcttctagtgtagccgtagttaggccaccacttcaagaactctgtagcaccgcctacatacctcgctctgctaatcctgttaccagtggctgctgccagtggcgataagtcgtgtcttaccgggttggactcaagacgatagttaccggataaggcgcagcggtcgggctgaacggggggttcgtgcacacagcccagcttggagcgaacgacctacaccgaactgagatacctacagcgtgagctatgagaaagcgccacgcttcccgaagggagaaaggcggacaggtatccggtaagcggcagggtcggaacaggagagcgcacgagggagcttccagggggaaacgcctggtatctttatagtcctgtcgggtttcgccacctctgacttgagcgtcgatttttgtgatgctcgtcaggggggcggagcctatggaaaaacgccagcaacgcggcctttttacggttcctggccttttgctggccttttgctcacatgttctttcctgcgttatcccctgattctgtggataaccgtattaccgcctttgagtgagctgataccgctcgccgcagccgaacgaccgagcgcagcgagtcagtgagcgaggaagcggaagagcgcccaatacgcaaaccgcctctccccgcgcgttggccgattcattaatgcagctggcacgacaggtttcccgactggaaagcgggcagtgagcgcaacgcaattaatgtgagttagctcactcattaggcaccccaggctttacactttatgcttccggctcgtatgttgtgtggaattgtgagcggataacaatttcacacaggaaacagctatgaccatgattacgcca

SEQ ID NO: 8 - DNA, 725 bp, Artificial Sequence
  cDNA encoding human omalizumab antibody light chain (OML) to be substitued for the sequence from No. 1267 to No. 1273 in pDC61
ggccgccaccatgggttggtcttgtatcatcttatttttagttgctactgctactggtgttcattctgatatacagctcacccaaagcccatcatctctgtctgcaagcgtcggcgacagggtgaccattacctgtcgcgcaagccaaagcgttgactacgacggcgacagctacatgaactggtaccagcagaagcccggcaaggctcctaagctgctgatctatgccgcctcctaccttgaatctggagtgccttctcgtttttccggctcagggtccggaactgattttaccctgaccatttcctccctccagcccgaggattttgccacttactactgtcagcagtcccacgaggacccatatacattcggacaaggtacaaaggtagaaatcaagcgtacggtggctgccccatccgtgttcatatttcctcctagcgacgaacaactcaagtccggtaccgccagcgtggtctgcctgttgaacaatttttatccaagagaagctaaggtccagtggaaggttgacaacgcccttcagtccggaaatagccaagagagcgtcaccgaacaggactccaaggacagtacatactcactgagctctacactgaccctttctaaggccgactacgagaagcacaaggtctacgcatgcgaagtgacccatcagggactcagtagccctgtaacaaagagttttaatcgaggcgagtgctaac

SEQ ID NO: 9 - DNA, 1423 bp, Artificial Sequence
  cDNA encoding human omalizumab antibody heavy chain (OMH) to be substitued for the sequence from No. 2765 to No. 2771 in pDC61
cgcgccaccatggaatttggtttatcttgggtttttttagttgctttattaagaggtgttcaatgtgaggtgcagttggtcgaatccggcggcggactcgtgcaaccaggcggaagtttgcggctgtcctgcgcagtgtctggttacagcatcacctccgggtatagctggaactggatccgccaggctcctggaaaggggcttgagtgggtggcttccattacctacgacggctccactaactataacccgagcgtcaaaggcagaatcaccatctctcgggacgactcaaagaataccttctacctgcagatgaactcactgagggccgaagataccgcagtttactactgcgccagggggtcccactatttcggccactggcacttcgccgtgtggggacagggcacactcgtgaccgttagtagcgctagcaccaaaggcccctctgtgttcccacttgctccctccagtaaatctacctccggaggaaccgcagccctcggctgcctggtgaaggattacttcccagagcccgtcaccgtctcttggaactccggagccttgactagcggagtgcacactttccctgctgtattgcagtccagcggcttgtattcactgagtagcgtcgtcaccgtgccttcaagcagcctcgggacacagacatacatatgtaatgtcaaccataagccatcaaacactaaagttgataaaaaggtggaacctaagagttgcgataagacccatacctgtcctccttgccctgctcctgagctgctgggaggccctagcgtgtttctgttcccccccaagcccaaagatacactgatgatttcccgcacacctgaagtaacatgtgtcgtggttgatgtgagtcacgaggatccagaggtcaagtttaattggtacgtggacggagtggaggtgcacaacgctaagactaagcctcgggaggaacagtacaacagcacataccgcgtggtcagcgttttgactgtgctgcatcaagactggctcaatggaaaggaatacaagtgcaaggtctctaataaagccctccccgctcctattgagaagactatttctaaagccaagggccagcctcgcgaacctcaggtatatactttgccaccctctcgcgaagaaatgacaaagaatcaggtctcactcacttgcctcgtcaaagggttttacccttctgacatcgctgtcgaatgggaaagtaatggtcagccagaaaacaattacaagactactccaccagtgctcgattctgatggaagtttctttctctacagtaagctcactgtggacaaatctcgctggcagcagggtaacgtattctcatgctccgtgatgcatgaagccctccacaaccattacacccagaagagcctgtctctgagcccaggcaagtaat

SEQ ID NO: 10 - DNA, 10686 bp, Artificial Sequence
  pNC32c-U533
cgatgtacgggccagatatacgcgttgacattgattattgactagttattaatagtaatcaattacggggtcattagttcatagcccatatatggagttccgcgttacataacttacggtaaatggcccgcctggctgaccgcccaacgacccccgcccattgacgtcaataatgacgtatgttcccatagtaacgccaatagggactttccattgacgtcaatgggtggagtatttacggtaaactgcccacttggcagtacatcaagtgtatcatatgccaagtacgccccctattgacgtcaatgacggtaaatggcccgcctggcattatgcccagtacatgaccttatgggactttcctacttggcagtacatctacgtattagtcatcgctattaccatggtgatgcggttttggcagtacatcaatgggcgtggatagcggtttgactcacggggatttccaagtctccaccccattgacgtcaatgggagtttgttttggcaccaaaatcaacgggactttccaaaatgtcgtaacaactccgccccattgacgcaaatgggcggtaggcgtgtacggtgggaggtctatataagcagagctctctggctaactagagaacccactgttaactggcttatcgaaattggcgcgccgcgatcgccctcccacacctccccctgaacctgaaacataaaatgaatgcaattgttgttgttaacttgtttattgcagcttataatggttacaaataaagcaatagcatcacaaatttcacaaataaagcatttttttcactgcattctagttgtggtttgtccaaactcatcaatgtatcttatcatgtctggatctccgcggccctccgcgcctacagctcaagccacatccgaagggggagggagccgggagctgcgcgcggggccgccggggggaggggtggcaccgcccacgccgggcggccacgaagggcggggcagcgggcgcgcgcgcggcggggggaggggccggcgccgcgcccgctgggaattggggccctagggggagggcggaggcgccgacgaccgcggcacttaccgttcgcggcgtggcgcccggtggtccccaaggggagggaagggggaggcggggcgaggacagtgaccggagtctcctcagcggtggcttttctgcttggcagcctcagcggctggcgccaaaaccggactccgcccacttcctcgcccgccggtgcgagggtgtggaatcctccagacgctgggggagggggagttgggagcttaaaaactagtacccctttgggaccactttcagcagcgaactctcctgtacaccaggggtcagttccacagacgcgggccaggggtgggtcattgcggcgtgaacaataatttgactagaagttgattcgggtgtttccggaaggggccgagtcaatccgccgagttggggcacggaaaacaaaaagggaaggctactaagatttttctggcgggggttatcattggcgtaactgcagggaccacctcccgggttgagggggctggatctccaggctgcggattaagcccctcccgtcggcgttaatttcaaactgcgcgacgtttctcacctgccttcgccaaggcaggggccgggaccctattccaagaggtagtaactagcaggactctagccttccgcaattcattgagcgcatttacggaagtaacgtcgggtactgtctctggccgcaagggtgggaggagtacgcatttggcgtaaggtggggcgtagagccttcccgccattggcggcggatagggcgtttacgcgacggcctgacgtagcggaagacgccttagtgggggggaaggttctagaaaagcggcggcagcggctctagcggcagtagcagcagcgccgggtcccgtgcggaggtgctcctcgcagagttgtttctccagcagcggcagttctcactacagcgccaggacgagtccggttcgtgttcgtccgcggagatctctctcatctcgctcggctgcgggaaatcgggctgaagcgactgagtccgcgatggaggtaacgggtttgaaatcaatgagttattgaaaagggcatggcgaggccgttggcgcctcagtggaagtcggccagccgcctccgtgggagagaggcaggaaatcggaccaattcagtagcagtggggcttaaggtttatgaacggggtcttgagcggaggcctgagcgtacaaacagcttccccaccctcagcctcccggcgccatttcccttcactgggggtgggggatggggagctttcacatggcggacgctgccccgctggggtgaaagtggggcgcggaggcgggacttcttattccctttctaaagcacgctgcttcgggggccacggcgtctcctcggagaattccgatgtacgggccagatatacgcgttgacattgattattgactagttattaatagtaatcaattacggggtcattagttcatagcccatatatggagttccgcgttacataacttacggtaaatggcccgcctggctgaccgcccaacgacccccgcccattgacgtcaataatgacgtatgttcccatagtaacgccaatagggactttccattgacgtcaatgggtggagtatttacggtaaactgcccacttggcagtacatcaagtgtatcatatgccaagtacgccccctattgacgtcaatgacggtaaatggcccgcctggcattatgcccagtacatgaccttatgggactttcctacttggcagtacatctacgtattagtcatcgctattaccatggtgatgcggttttggcagtacatcaatgggcgtggatagcggtttgactcacggggatttccaagtctccaccccattgacgtcaatgggagtttgttttggcaccaaaatcaacgggactttccaaaatgtcgtaacaactccgccccattgacgcaaatgggcggtaggcgtgtacggtgggaggtctatataagcagagctctctggctaactagagaacccactgttaactggcttatcgaaattgcggccgccctgcaggcctcccacacctccccctgaacctgaaacataaaatgaatgcaattgttgttgttaacttgtttattgcagcttataatggttacaaataaagcaatagcatcacaaatttcacaaataaagcatttttttcactgcattctagttgtggtttgtccaaactcatcaatgtatcttatcatgtctggactccgcggggccctccgcgcctacagctcaagccacatccgaagggggagggagccgggagctgcgcgcggggccgccggggggaggggtggcaccgcccacgccgggcggccacgaagggcggggcagcgggcgcgcgcgcggcggggggaggggccggcgccgcgcccgctgggaattggggccctagggggagggcggaggcgccgacgaccgcggcacttaccgttcgcggcgtggcgcccggtggtccccaaggggagggaagggggaggcggggcgaggacagtgaccggagtctcctcagcggtggcttttctgcttggcagcctcagcggctggcgccaaaaccggactccgcccacttcctcgcccgccggtgcgagggtgtggaatcctccagacgctgggggagggggagttgggagcttaaaaactagtacccctttgggaccactttcagcagcgaactctcctgtacaccaggggtcagttccacagacgcgggccaggggtgggtcattgcggcgtgaacaataatttgactagaagttgattcgggtgtttccggaaggggccgagtcaatccgccgagttggggcacggaaaacaaaaagggaaggctactaagatttttctggcgggggttatcattggcgtaactgcagggaccacctcccgggttgagggggctggatctccaggctgcggattaagcccctcccgtcggcgttaatttcaaactgcgcgacgtttctcacctgccttcgccaaggcaggggccgggaccctattccaagaggtagtaactagcaggactctagccttccgcaattcattgagcgcatttacggaagtaacgtcgggtactgtctctggccgcaagggtgggaggagtacgcatttggcgtaaggtggggcgtagagccttcccgccattggcggcggatagggcgtttacgcgacggcctgacgtagcggaagacgccttagtgggggggaaggttctagaaaagcggcggcagcggctctagcggcagtagcagcagcgccgggtcccgtgcggaggtgctcctcgcagagttgtttctccagcagcggcagttctcactacagcgccaggacgagtccggttcgtgttcgtccgcggagatctctctcatctcgctcggctgcgggaaatcgggctgaagcgactgagtccgcgatggaggtaacgggtttgaaatcaatgagttattgaaaagggcatggcgaggccgttggcgcctcagtggaagtcggccagccgcctccgtgggagagaggcaggaaatcggaccaattcagtagcagtggggcttaaggtttatgaacggggtcttgagcggaggcctgagcgtacaaacagcttccccaccctcagcctcccggcgccatttcccttcactgggggtgggggatggggagctttcacatggcggacgctgccccgctggggtgaaagtggggcgcggaggcgggacttcttattccctttctaaagcacgctgcttcgggggccacggcgtctcctcggaaccggttgtggaatgtgtgtcagttagggtgtggaaagtccccaggctccccagcaggcagaagtatgcaaagcatgcatctcaattagtcagcaaccaggtgtggaaagtccccaggctccccagcaggcagaagtatgcaaagcatgcatctcaattagtcagcaaccatagtcccgcccctaactccgcccatcccgcccctaactccgcccagttccgcccattctccgccccatggctgactaattttttttatttatgcagaggccgaggccgcctcggcctctgagctattccagaagtagtgaggaggcttttttggaggcctaggcttttgcaaaaaagctgcagatgattgaacaagatggattgcacgcaggttctccggccgcttgggtggagaggctattcggctatgactgggcacaacagacaatcggctgctctgatgccgccgtgttccggctgtcagcgcaggggcgcccggttctttttgtcaagaccgacctgtccggtgccctgaatgaactgcaggacgaggcagcgcggctatcgtggctggccacgacgggcgttccttgcgcagctgtgctcgacgttgtcactgaagcgggaagggactggctgctattgggcgaagtgccggggcaggatctcctgtcatctcaccttgctcctgccgagaaagtatccatcatggctgatgcaatgcggcggctgcatacgcttgatccggctacctgcccattcgaccaccaagcgaaacatcgcatcgagcgagcacgtactcggatggaagccggtcttgtcgatcaggatgatctggacgaagagcatcaggggctcgcgccagccgaactgttcgccaggctcaaggcgcgcatgcccgacggcgaggatctcgtcgtgacccatggcgatgcctgcttgccgaatatcatggtggaaaatggccgcttttctggattcatcgactgtggccggctgggtgtggcggaccgctatcaggacatagcgttggctacccgtgatattgctgaagagcttggcggcgaatgggctgaccgcttcctcgtgctttacggtatcgccgctcccgattcgcagcgcatcgccttctatcgccttcttgacgagttcttctgagatccgtgacataattggacaaactacctacagagatttaaagctctaaggtaaatataaaatttttaagtgtataatgtgttaaactactgattctaattgtttgtgtattttagattccaacctatggaactgatgaatgggagcagtggtggaatgcctttaatgaggaaaacctgttttgctcagaagaaatgccatctagtgatgatgaggctactgctgactctcaacattctactcctccaaaaaagaagagaaaggtagaagaccccaaggactttccttcagaattgctaagttttttgagtcatgctgtgtttagtaatagaactcttgcttgctttgctatttacaccacaaaggaaaaagctgcactgctatacaagaaaattatggaaaaatattctgtaacctttataagtaggcataacagttataatcataacatactgttttttcttactccacacaggcatagagtgtctgctattaataactatgctcaaaaattgtgtacctttagctttttaatttgtaaaggggttaataaggaatatttgatgtatagtgccttgactagagatcataatcagccataccacatttgtagaggttttacttgctttaaaaaacctcccacacctccccctgaacctgaaacataaaatgaatgcaattgttgttgttaacttgtttattgcagcttataatggttacaaataaagcaatagcatcacaaatttcacaaataaagcatttttttcactgcattctagttgtggtttgtccaaactcatcaatgtatcttatcatgtctgggcccatcgatgccgacgtagcgcctgatgcggtattttctccttacgcatctgtgcggtatttcacaccgcatatggtgcactctcagtacaatctgctctgatgccgcatagttaagccagccccgacacccgccaacacccgctgacgcgccctgacgggcttgtctgctcccggcatccgcttacagacaagctgtgaccgtctccgggagctgcatgtgtcagaggttttcaccgtcatcaccgaaacgcgcgagacgaaagggcctcgtgatacgcctatttttataggttaatgtcatgataataatggtttcttagacgtcaggtggcacttttcggggaaatgtgcgcggaacccctatttgtttatttttctaaatacattcaaatatgtatccgctcatgagacaataaccctgataaatgcttcaataatattgaaaaaggaagagtatgagtattcaacatttccgtgtcgcccttattcccttttttgcggcattttgccttcctgtttttgctcacccagaaacgctggtgaaagtaaaagatgctgaagatcagttgggtgcacgagtgggttacatcgaactggatctcaacagcggtaagatccttgagagttttcgccccgaagaacgttttccaatgatgagcacttttaaagttctgctatgtggcgcggtattatcccgtattgacgccgggcaagagcaactcggtcgccgcatacactattctcagaatgacttggttgagtactcaccagtcacagaaaagcatcttacggatggcatgacagtaagagaattatgcagtgctgccataaccatgagtgataacactgcggccaacttacttctgacaacgatcggaggaccgaaggagctaaccgcttttttgcacaacatgggggatcatgtaactcgccttgatcgttgggaaccggagctgaatgaagccataccaaacgacgagcgtgacaccacgatgcctgtagcaatggcaacaacgttgcgcaaactattaactggcgaactacttactctagcttcccggcaacaattaatagactggatggaggcggataaagttgcaggaccacttctgcgctcggcccttccggctggctggtttattgctgataaatctggagccggtgagcgtgggtctcgcggtatcattgcagcactggggccagatggtaagccctcccgtatcgtagttatctacacgacggggagtcaggcaactatggatgaacgaaatagacagatcgctgagataggtgcctcactgattaagcattggtaactgtcagaccaagtttactcatatatactttagattgatttaaaacttcatttttaatttaaaaggatctaggtgaagatcctttttgataatctcatgaccaaaatcccttaacgtgagttttcgttccactgagcgtcagaccccgtagaaaagatcaaaggatcttcttgagatcctttttttctgcgcgtaatctgctgcttgcaaacaaaaaaaccaccgctaccagcggtggtttgtttgccggatcaagagctaccaactctttttccgaaggtaactggcttcagcagagcgcagataccaaatactgttcttctagtgtagccgtagttaggccaccacttcaagaactctgtagcaccgcctacatacctcgctctgctaatcctgttaccagtggctgctgccagtggcgataagtcgtgtcttaccgggttggactcaagacgatagttaccggataaggcgcagcggtcgggctgaacggggggttcgtgcacacagcccagcttggagcgaacgacctacaccgaactgagatacctacagcgtgagctatgagaaagcgccacgcttcccgaagggagaaaggcggacaggtatccggtaagcggcagggtcggaacaggagagcgcacgagggagcttccagggggaaacgcctggtatctttatagtcctgtcgggtttcgccacctctgacttgagcgtcgatttttgtgatgctcgtcaggggggcggagcctatggaaaaacgccagcaacgcggcctttttacggttcctggccttttgctggccttttgctcacatgttctttcctgcgttatcccctgattctgtggataaccgtattaccgcctttgagtgagctgataccgctcgccgcagccgaacgaccgagcgcagcgagtcagtgagcgaggaagcggaagagcgcccaatacgcaaaccgcctctccccgcgcgttggccgattcattaatgcagctgggccctccgcgcctacagctcaagccacatccgaagggggagggagccgggagctgcgcgcggggccgccggggggaggggtggcaccgcccacgccgggcggccacgaagggcggggcagcgggcgcgcgcgcggcggggggaggggccggcgccgcgcccgctgggaattggggccctagggggagggcggaggcgccgacgaccgcggcacttaccgttcgcggcgtggcgcccggtggtccccaaggggagggaagggggaggcggggcgaggacagtgaccggagtctcctcagcggtggcttttctgcttggcagcctcagcggctggcgccaaaaccggactccgcccacttcctcgcccgccggtgcgagggtgtggaatcctccagacgctgggggagggggagttgggagcttaaaaactagtacccctttgggaccactttcagcagcgaactctcctgtacaccaggggtcagttccacagacgcgggccaggggtgggtcattgcggcgtgaacaataatttgactagaagttgattcgggtgtttccggaaggggccgagtcaatccgccgagttggggcacggaaaacaaaaagggaaggctactaagatttttctggcgggggttatcattggcgtaactgcagggaccacctcccgggttgagggggctggatctccaggctgcggattaagcccctcccgtcggcgttaatttcaaactgcgcgacgtttctcacctgccttcgccaaggcaggggccgggaccctattccaagaggtagtaactagcaggactctagccttccgcaattcattgagcgcatttacggaagtaacgtcgggtactgtctctggccgcaagggtgggaggagtacgcatttggcgtaaggtggggcgtagagccttcccgccattggcggcggatagggcgtttacgcgacggcctgacgtagcggaagacgccttagtgggggggaaggttctagaaaagcggcggcagcggctctagcggcagtagcagcagcgccgggtcccgtgcggaggtgctcctcgcagagttgtttctccagcagcggcagttctcactacagcgccaggacgagtccggttcgtgttcgtccgcggagatctctctcatctcgctcggctgcgggaaatcgggctgaagcgactgagtccgcgatggaggtaacgggtttgaaatcaatgagttattgaaaagggcatggcgaggccgttggcgcctcagtggaagtcggccagccgcctccgtgggagagaggcaggaaatcggaccaattcagtagcagtggggcttaaggtttatgaacggggtcttgagcggaggcctgagcgtacaaacagcttccccaccctcagcctcccggcgccatttcccttcactgggggtgggggatggggagctttcacatggcggacgctgccccgctggggtgaaagtggggcgcggaggcgggacttcttattccctttctaaagcacgctgcttcgggggccacggcgtctcctcggaaagctt

SEQ ID NO: 11 - DNA, 728 bp, Artificial Sequence
  cDNA encoding human omalizumab antibody (OKLH) light chain to be substitued for the sequence from No. 658 to No. 668 in pNC32c-U533
cgcgccaccatgggttggtcttgtatcatcttatttttagttgctactgctactggtgttcattctgatatacagctcacccaaagcccatcatctctgtctgcaagcgtcggcgacagggtgaccattacctgtcgcgcaagccaaagcgttgactacgacggcgacagctacatgaactggtaccagcagaagcccggcaaggctcctaagctgctgatctatgccgcctcctaccttgaatctggagtgccttctcgtttttccggctcagggtccggaactgattttaccctgaccatttcctccctccagcccgaggattttgccacttactactgtcagcagtcccacgaggacccatatacattcggacaaggtacaaaggtagaaatcaagcgtacggtggctgccccatccgtgttcatatttcctcctagcgacgaacaactcaagtccggtaccgccagcgtggtctgcctgttgaacaatttttatccaagagaagctaaggtccagtggaaggttgacaacgcccttcagtccggaaatagccaagagagcgtcaccgaacaggactccaaggacagtacatactcactgagctctacactgaccctttctaaggccgactacgagaagcacaaggtctacgcatgcgaagtgacccatcagggactcagtagccctgtaacaaagagttttaatcgaggcgagtgctaagcgat

SEQ ID NO: 12 - DNA, 1429 bp, Artificial Sequence
  cDNA encoding human omalizumab antibody (OKLH) heavy chain to be substitued for the sequence from No. 3081 to No. 3092 in pNC32c-U533
ggccgccaccatggaatttggtttatcttgggtttttttagttgctttattaagaggtgttcaatgtgaggtgcagttggtcgaatccggcggcggactcgtgcaaccaggcggaagtttgcggctgtcctgcgcagtgtctggttacagcatcacctccgggtatagctggaactggatccgccaggctcctggaaaggggcttgagtgggtggcttccattacctacgacggctccactaactataacccgagcgtcaaaggcagaatcaccatctctcgggacgactcaaagaataccttctacctgcagatgaactcactgagggccgaagataccgcagtttactactgcgccagggggtcccactatttcggccactggcacttcgccgtgtggggacagggcacactcgtgaccgttagtagcgctagcaccaaaggcccctctgtgttcccacttgctccctccagtaaatctacctccggaggaaccgcagccctcggctgcctggtgaaggattacttcccagagcccgtcaccgtctcttggaactccggagccttgactagcggagtgcacactttccctgctgtattgcagtccagcggcttgtattcactgagtagcgtcgtcaccgtgccttcaagcagcctcgggacacagacatacatatgtaatgtcaaccataagccatcaaacactaaagttgataaaaaggtggaacctaagagttgcgataagacccatacctgtcctccttgccctgctcctgagctgctgggaggccctagcgtgtttctgttcccccccaagcccaaagatacactgatgatttcccgcacacctgaagtaacatgtgtcgtggttgatgtgagtcacgaggatccagaggtcaagtttaattggtacgtggacggagtggaggtgcacaacgctaagactaagcctcgggaggaacagtacaacagcacataccgcgtggtcagcgttttgactgtgctgcatcaagactggctcaatggaaaggaatacaagtgcaaggtctctaataaagccctccccgctcctattgagaagactatttctaaagccaagggccagcctcgcgaacctcaggtatatactttgccaccctctcgcgaagaaatgacaaagaatcaggtctcactcacttgcctcgtcaaagggttttacccttctgacatcgctgtcgaatgggaaagtaatggtcagccagaaaacaattacaagactactccaccagtgctcgattctgatggaagtttctttctctacagtaagctcactgtggacaaatctcgctggcagcagggtaacgtattctcatgctccgtgatgcatgaagccctccacaaccattacacccagaagagcctgtctctgagcccaggcaagtaacctgca

SEQ ID NO: 13 - DNA, 24 bp, Artificial Sequence
  BstBI recognition site-containing sequence to be substituted for the sequence from No. 5309 to No. 5311 in UCOE-Hu-P
cctagtagtagtagtagttcgaag

SEQ ID NO: 14 - DNA, 3400 bp, Artificial Sequence
  cDNA encoding human omalizumab antibody light chain (OML) linking to cDNA encoding Simian Virus 40 polyadenylation signal (SV40pA), guinea pig cytomegalovirus promoter (PgpCMV) and human omalizumab antibody heavy chain (OMH)
cccaccatgggttggtcttgtatcatcttatttttagttgctactgctactggtgttcattctgatatacagctcacccaaagcccatcatctctgtctgcaagcgtcggcgacagggtgaccattacctgtcgcgcaagccaaagcgttgactacgacggcgacagctacatgaactggtaccagcagaagcccggcaaggctcctaagctgctgatctatgccgcctcctaccttgaatctggagtgccttctcgtttttccggctcagggtccggaactgattttaccctgaccatttcctccctccagcccgaggattttgccacttactactgtcagcagtcccacgaggacccatatacattcggacaaggtacaaaggtagaaatcaagcgtacggtggctgccccatccgtgttcatatttcctcctagcgacgaacaactcaagtccggtaccgccagcgtggtctgcctgttgaacaatttttatccaagagaagctaaggtccagtggaaggttgacaacgcccttcagtccggaaatagccaagagagcgtcaccgaacaggactccaaggacagtacatactcactgagctctacactgaccctttctaaggccgactacgagaagcacaaggtctacgcatgcgaagtgacccatcagggactcagtagccctgtaacaaagagttttaatcgaggcgagtgctaagcgatcgcgctagcgcggccacgtagtcgactacgtagagctcggtacccggggatcctctagagtcgacctgcaggcatgcaagctggccgcgactctagatcataatcagccataccacatttgtagaggttttacttgctttaaaaaacctcccacacctccccctgaacctgaaacataaaatgaatgcaattgttgttgttaacttgtttattgcagcttataatggttacaaataaagcaatagcatcacaaatttcacaaataaagcatttttttcactgcattctagttgtggtttgtccaaactcatcaatgtatcttaaccggttatgttacttggcagaggccgcatggaaagtccctggacgtgggacatctgattaatacgtgaggaggtcagccatgttctttttggcaaaggactacggtcattggacgtttgattggcatgggatagggtcagccagagttaacagtgttcttttggcaaagggatacgtggaaagtcccgggccatttacagtaaactgatacggggacaaagcacagccatatttagtcatgtattgcttggcagagggtctatggaaagtccctggacgtgggacgtctgattaatatgaaagaaggtcagccagaggtagctgtgtcctttttggcaaagggatacggttatgggacgtttgattggactgggatagggtcagccagagttaacagtgttcttttggcaaaggaaacgtggaaagtcccgggccatttacagtaaactgatactgggacaaagtacacccatatttagtcatgttctttttggcaaagagcatctggaaagtcccgggcagcattatagtcacttggcagagggaaagggtcactcagagttaagtacatctttccagggccaatattccagtaaattacacttagttttatgcaaatcagccacaaaggggattttcccggtcaattatgactttttccttagtcatgcggtatccaattactgccaaattggcagtacatactaggtgattcactgacatttggccgtcctctggaaagtccctggaaaccgctcaagtactgtatcatggtgactttgcatttttggagagcacgccccactccaccattggtccacgtaccctatgggggagtggtttatgagtatataaggggctccggtttagaagccgggcagagcggaattcgagctccctgcaggttagttaagttaacggcgcgccaccatggaatttggtttatcttgggtttttttagttgctttattaagaggtgttcaatgtgaggtgcagttggtcgaatccggcggcggactcgtgcaaccaggcggaagtttgcggctgtcctgcgcagtgtctggttacagcatcacctccgggtatagctggaactggatccgccaggctcctggaaaggggcttgagtgggtggcttccattacctacgacggctccactaactataacccgagcgtcaaaggcagaatcaccatctctcgggacgactcaaagaataccttctacctgcagatgaactcactgagggccgaagataccgcagtttactactgcgccagggggtcccactatttcggccactggcacttcgccgtgtggggacagggcacactcgtgaccgttagtagcgctagcaccaaaggcccctctgtgttcccacttgctccctccagtaaatctacctccggaggaaccgcagccctcggctgcctggtgaaggattacttcccagagcccgtcaccgtctcttggaactccggagccttgactagcggagtgcacactttccctgctgtattgcagtccagcggcttgtattcactgagtagcgtcgtcaccgtgccttcaagcagcctcgggacacagacatacatatgtaatgtcaaccataagccatcaaacactaaagttgataaaaaggtggaacctaagagttgcgataagacccatacctgtcctccttgccctgctcctgagctgctgggaggccctagcgtgtttctgttcccccccaagcccaaagatacactgatgatttcccgcacacctgaagtaacatgtgtcgtggttgatgtgagtcacgaggatccagaggtcaagtttaattggtacgtggacggagtggaggtgcacaacgctaagactaagcctcgggaggaacagtacaacagcacataccgcgtggtcagcgttttgactgtgctgcatcaagactggctcaatggaaaggaatacaagtgcaaggtctctaataaagccctccccgctcctattgagaagactatttctaaagccaagggccagcctcgcgaacctcaggtatatactttgccaccctctcgcgaagaaatgacaaagaatcaggtctcactcacttgcctcgtcaaagggttttacccttctgacatcgctgtcgaatgggaaagtaatggtcagccagaaaacaattacaagactactccaccagtgctcgattctgatggaagtttctttctctacagtaagctcactgtggacaaatctcgctggcagcagggtaacgtattctcatgctccgtgatgcatgaagccctccacaaccattacacccagaagagcctgtctctgagcccaggcaagtaatctagatt

SEQ ID NO: 15 - protein, 394 aa, Canis lupus
MAGFGFRRHGAQPDLASRTWPCTALFSLLFIPVFSKGMHVAQPAVVLASSRGVASFVCEYGSSGNAAEVRVTVLRQAGSQMTEVCAATYTVEDELAFLDDSTCTGTSSGNKVNLTIQGLRAMDTGLYICKVELMYPPPYYVGMGNGTQIYVIDPEPCPDSDPKESTCKCISPCPVPESLGGPSVFIFPPKPKDILRITRTPEITCVVLDLGREDPEVQISWFVDGKEVHTAKTQPREQQFNSTYRVVSVLPIEHQDWLTGKEFKCRVNHIGLPSPIERTISKARGQAHQPSVYVLPPSPKELSSSDTVTLTCLIKDFFPPEIDVEWQSNGQPEPESKYHTTAPQLDEDGSYFLYSKLSVDKSRWQQGDTFTCAVMHEALQNHYTDLSLSHSPGK

SEQ ID NO: 16 - DNA, 1185 bp, Artificial Sequence
  Codon-optimized nucleotide sequence encoding canis lupus CTLA-4-Ig
atggctggatttggattcagaaggcacggagcccagcccgacctggcatctcgcacttggccctgtaccgcactgttttcactgctgttcatcccagtgttcagcaagggaatgcacgtggctcagccagctgtggtgctggcttccagcagaggcgtggcttccttcgtgtgcgagtacggctcttccggcaacgccgctgaggtgagagtgaccgtgctgaggcaggctggctcccagatgacagaggtgtgcgccgctacctatacagtggaggacgagctggctttcctggacgatagcacctgtacaggcaccagctctggcaacaaggtcaatctgaccatccagggcctgcgcgccatggatacaggcctgtacatctgtaaggtggagctgatgtatccccctccatactatgtgggcatgggcaatggcacccagatctacgtgatcgaccccgagccttgcccagactctgatccaaaggagtcgacatgcaagtgtatctctccatgtcctgtgccagagagcctgggaggaccttccgtgttcatctttccccctaagccaaaggatatcctgaggatcacacggacccctgagatcacctgcgtggtgctggacctgggaagggaggatccagaggtgcagatctcctggttcgtggacggcaaggaggtgcataccgctaagacacagcccagagagcagcagtttaactccacctatcgcgtggtgagcgtgctgcctatcgagcaccaggattggctgacaggcaaggagtttaagtgccgggtgaatcatatcggcctgccctctcctatcgagaggaccatctccaaggctaggggacaggctcaccagccaagcgtgtacgtgctgccaccctctcctaaggagctgtccagctctgacacagtgaccctgacatgtctgatcaaggacttctttcctccagagatcgacgtggagtggcagtccaacggccagccagagcccgagagcaagtatcataccacagccccccagctggacgaggatggctcttacttcctgtattccaagctgagcgtggacaagtccaggtggcagcagggcgatacctttacatgtgctgtgatgcacgaagccctgcagaatcattacaccgacctgtcactgtcccactcccctggcaaataa

SEQ ID NO: 17 - DNA, 8444 bp, Artificial Sequence
  pDC62c5-U533 containing one cloning site
cgatgtacgggccagatatacgcgttgacattgattattgactagtcgcgttacataacttacggtaaatggcccgcctggctgaccgcccaacgacccccgcccattgacgtcaataatgacgtatgttcccatagtaacgccaatagggactttccattgacgtcaatgggtggagtatttacggtaaactgcccacttggcagtacatcaagtgtatcatatgccaagtccgccccctattgacgtcaatgacggtaaatggcccgcctggcattatgcccagtacatgaccttacgggactttcctacttggcagtacatctacgtattagtcatcgctattaccatggtgatgcggttttggcagtacaccaatgggcgtggatagcggtttgactcacggggatttccaagtctccaccccattgacgtcaatgggagtttgttttggcaccaaaatcaacgggactttccaaaatgtcgtaataaccccgccccgttgacgcaaatgggcggtaggcgtgtacggtgggaggtctatataagcagagctcgtttagtgaaccgtcagatcctcactctcttccgcatcgctgtctgcgagggccagctgttgggctcgcggttgaggacaaactcttcgcggtctttccagtactcttggatcggaaacccgtcggcctccgaacggtactccgccaccgagggacctgagcgagtccgcatcgaccggatcggaaaacctctcgagaaaggcgtctaaccagtcacagtcgcaaggtaggctgagcaccgtggcgggcggcagcgggtggcggtcggggttgtttctggcggaggtgctgctgatgatgtaattaaagtaggcggtcttgagacggcggatggtcgaggtgaggtgtggcaggcttgagatccagctgttggggtgagtactccctctcaaaagcgggcatgacttctgcgctaagattgtcagtttccaaaaacgaggaggatttgatattcacctggcccgatctggccatacacttgagtgacaatgacatccactttgcctttctctccacaggtgtccactcccaggtccaaggcgcgccgcgatcgcgcctcgactgtgccttctagttgccagccatctgttgtttgcccctcccccgtgccttccttgaccctggaaggtgccactcccactgtcctttcctaataaaatgaggaaattgcatcgcattgtctgagtaggtgtcattctattctggggggtggggtggggcaggacagcaagggggaggattgggaagacaatagcaggcatgctggggaggatctccgcggggccctccgcgcctacagctcaagccacatccgaagggggagggagccgggagctgcgcgcggggccgccggggggaggggtggcaccgcccacgccgggcggccacgaagggcggggcagcgggcgcgcgcgcggcggggggaggggccggcgccgcgcccgctgggaattggggccctagggggagggcggaggcgccgacgaccgcggcacttaccgttcgcggcgtggcgcccggtggtccccaaggggagggaagggggaggcggggcgaggacagtgaccggagtctcctcagcggtggcttttctgcttggcagcctcagcggctggcgccaaaaccggactccgcccacttcctcgcccgccggtgcgagggtgtggaatcctccagacgctgggggagggggagttgggagcttaaaaactagtacccctttgggaccactttcagcagcgaactctcctgtacaccaggggtcagttccacagacgcgggccaggggtgggtcattgcggcgtgaacaataatttgactagaagttgattcgggtgtttccggaaggggccgagtcaatccgccgagttggggcacggaaaacaaaaagggaaggctactaagatttttctggcgggggttatcattggcgtaactgcagggaccacctcccgggttgagggggctggatctccaggctgcggattaagcccctcccgtcggcgttaatttcaaactgcgcgacgtttctcacctgccttcgccaaggcaggggccgggaccctattccaagaggtagtaactagcaggactctagccttccgcaattcattgagcgcatttacggaagtaacgtcgggtactgtctctggccgcaagggtgggaggagtacgcatttggcgtaaggtggggcgtagagccttcccgccattggcggcggatagggcgtttacgcgacggcctgacgtagcggaagacgccttagtgggggggaaggttctagaaaagcggcggcagcggctctagcggcagtagcagcagcgccgggtcccgtgcggaggtgctcctcgcagagttgtttctccagcagcggcagttctcactacagcgccaggacgagtccggttcgtgttcgtccgcggagatctctctcatctcgctcggctgcgggaaatcgggctgaagcgactgagtccgcgatggaggtaacgggtttgaaatcaatgagttattgaaaagggcatggcgaggccgttggcgcctcagtggaagtcggccagccgcctccgtgggagagaggcaggaaatcggaccaattcagtagcagtggggcttaaggtttatgaacggggtcttgagcggaggcctgagcgtacaaacagcttccccaccctcagcctcccggcgccatttcccttcactgggggtgggggatggggagctttcacatggcggacgctgccccgctggggtgaaagtggggcgcggaggcgggacttcttattccctttctaaagcacgctgcttcgggggccacggcgtctcctcggagaattcaaatgggaccggttgtggaatgtgtgtcagttagggtgtggaaagtccccaggctccccagcaggcagaagtatgcaaagcatgcatctcaattagtcagcaaccatagtcccgcccctaactccgcccatcccgcccctaactccgcccagttccgcccattctccgccccatggctgactaattttttttatttatgcagaggccgaggccgcctcggcctctgagctattccagaagtagtgaggaggcttttttggaggcctaggcttttgcaaaaaagctgcagatggtacgaccattaaattgtattgtagcagtatcacaaaatatgggtattggtaaaaatggtgatttaccatggccaccattacgaaatgaatttaaatattttcaacgaatgactactacttcatcagtagaaggtaaacaaaatttagtaattatgggtcgaaaaacttggttttcaattcctgagaagaatcgacctttaaaggacagaattaatatagttctcagtagagaactcaaagaaccaccacgaggagctcattttcttgccaaaagtttggatgatgccttaagacttattgaacaaccggaattggcaagtaaagtagacatggtttggatagtcggaggcagttctgtttaccaggaagccatgaatcaaccaggccacctcagactctttgtgacaaggatcatgcaggaatttgaaagtgacacgtttttcccagaaattgatttggggaaatataaacttctcccagaatacccaggcgtcctctctgaggtccaggaggaaaaaggcatcaagtataagtttgaagtctacgagaagaaagactaaagatccgtgacataattggacaaactacctacagagatttaaagctctaaggtaaatataaaatttttaagtgtataatgtgttaaactactgattctaattgtttgtgtattttagattccaacctatggaactgatgaatgggagcagtggtggaatgcctttaatgaggaaaacctgttttgctcagaagaaatgccatctagtgatgatgaggctactgctgactctcaacattctactcctccaaaaaagaagagaaaggtagaagaccccaaggactttccttcagaattgctaagttttttgagtcatgctgtgtttagtaatagaactcttgcttgctttgctatttacaccacaaaggaaaaagctgcactgctatacaagaaaattatggaaaaatattctgtaacctttataagtaggcataacagttataatcataacatactgttttttcttactccacacaggcatagagtgtctgctattaataactatgctcaaaaattgtgtacctttagctttttaatttgtaaaggggttaataaggaatatttgatgtatagtgccttgactagagatcataatcagccataccacatttgtagaggttttacttgctttaaaaaacctcccacacctccccctgaacctgaaacataaaatgaatgcaattgttgttgttaacttgtttattgcagcttataatggttacaaataaagcaatagcatcacaaatttcacaaataaagcatttttttcactgcattctagttgtggtttgtccaaactcatcaatgtatcttatcatgtctgggcccatcgatgccgacgtagcgctgatgcggtattttctccttacgcatctgtgcggtatttcacaccgcatatggtgcactctcagtacaatctgctctgatgccgcatagttaagccagccccgacacccgccaacacccgctgacgcgccctgacgggcttgtctgctcccggcatccgcttacagacaagctgtgaccgtctccgggagctgcatgtgtcagaggttttcaccgtcatcaccgaaacgcgcgagacgaaagggcctcgtgatacgcctatttttataggttaatgtcatgataataatggtttcttagacgtcaggtggcacttttcggggaaatgtgcgcggaacccctatttgtttatttttctaaatacattcaaatatgtatccgctcatgagacaataaccctgataaatgcttcaataatattgaaaaaggaagagtatgagtattcaacatttccgtgtcgcccttattcccttttttgcggcattttgccttcctgtttttgctcacccagaaacgctggtgaaagtaaaagatgctgaagatcagttgggtgcacgagtgggttacatcgaactggatctcaacagcggtaagatccttgagagttttcgccccgaagaacgttttccaatgatgagcacttttaaagttctgctatgtggcgcggtattatcccgtattgacgccgggcaagagcaactcggtcgccgcatacactattctcagaatgacttggttgagtactcaccagtcacagaaaagcatcttacggatggcatgacagtaagagaattatgcagtgctgccataaccatgagtgataacactgcggccaacttacttctgacaacgatcggaggaccgaaggagctaaccgcttttttgcacaacatgggggatcatgtaactcgccttgatcgttgggaaccggagctgaatgaagccataccaaacgacgagcgtgacaccacgatgcctgtagcaatggcaacaacgttgcgcaaactattaactggcgaactacttactctagcttcccggcaacaattaatagactggatggaggcggataaagttgcaggaccacttctgcgctcggcccttccggctggctggtttattgctgataaatctggagccggtgagcgtgggtctcgcggtatcattgcagcactggggccagatggtaagccctcccgtatcgtagttatctacacgacggggagtcaggcaactatggatgaacgaaatagacagatcgctgagataggtgcctcactgattaagcattggtaactgtcagaccaagtttactcatatatactttagattgatttaaaacttcatttttaatttaaaaggatctaggtgaagatcctttttgataatctcatgaccaaaatcccttaacgtgagttttcgttccactgagcgtcagaccccgtagaaaagatcaaaggatcttcttgagatcctttttttctgcgcgtaatctgctgcttgcaaacaaaaaaaccaccgctaccagcggtggtttgtttgccggatcaagagctaccaactctttttccgaaggtaactggcttcagcagagcgcagataccaaatactgttcttctagtgtagccgtagttaggccaccacttcaagaactctgtagcaccgcctacatacctcgctctgctaatcctgttaccagtggctgctgccagtggcgataagtcgtgtcttaccgggttggactcaagacgatagttaccggataaggcgcagcggtcgggctgaacggggggttcgtgcacacagcccagcttggagcgaacgacctacaccgaactgagatacctacagcgtgagcattgagaaagcgccacgcttcccgaagggagaaaggcggacaggtatccggtaagcggcagggtcggaacaggagagcgcacgagggagcttccagggggaaacgcctggtatctttatagtcctgtcgggtttcgccacctctgacttgagcgtcgatttttgtgatgctcgtcaggggggcggagcctatggaaaaacgccagcaacgcggcctttttacggttcctggccttttgctggccttttgctcacatgttctttcctgcgttatcccctgattctgtggataaccgtattaccgcctttgagtgagctgataccgctcgccgcagccgaacgaccgagcgcagcgagtcagtgagcgaggaagcggaagagcgcccaatacgcaaaccgcctctccccgcgcgttggccgattcattaatgcagctgggccctccgcgcctacagctcaagccacatccgaagggggagggagccgggagctgcgcgcggggccgccggggggaggggtggcaccgcccacgccgggcggccacgaagggcggggcagcgggcgcgcgcgcggcggggggaggggccggcgccgcgcccgctgggaattggggccctagggggagggcggaggcgccgacgaccgcggcacttaccgttcgcggcgtggcgcccggtggtccccaaggggagggaagggggaggcggggcgaggacagtgaccggagtctcctcagcggtggcttttctgcttggcagcctcagcggctggcgccaaaaccggactccgcccacttcctcgcccgccggtgcgagggtgtggaatcctccagacgctgggggagggggagttgggagcttaaaaactagtacccctttgggaccactttcagcagcgaactctcctgtacaccaggggtcagttccacagacgcgggccaggggtgggtcattgcggcgtgaacaataatttgactagaagttgattcgggtgtttccggaaggggccgagtcaatccgccgagttggggcacggaaaacaaaaagggaaggctactaagatttttctggcgggggttatcattggcgtaactgcagggaccacctcccgggttgagggggctggatctccaggctgcggattaagcccctcccgtcggcgttaatttcaaactgcgcgacgtttctcacctgccttcgccaaggcaggggccgggaccctattccaagaggtagtaactagcaggactctagccttccgcaattcattgagcgcatttacggaagtaacgtcgggtactgtctctggccgcaagggtgggaggagtacgcatttggcgtaaggtggggcgtagagccttcccgccattggcggcggatagggcgtttacgcgacggcctgacgtagcggaagacgccttagtgggggggaaggttctagaaaagcggcggcagcggctctagcggcagtagcagcagcgccgggtcccgtgcggaggtgctcctcgcagagttgtttctccagcagcggcagttctcactacagcgccaggacgagtccggttcgtgttcgtccgcggagatctctctcatctcgctcggctgcgggaaatcgggctgaagcgactgagtccgcgatggaggtaacgggtttgaaatcaatgagttattgaaaagggcatggcgaggccgttggcgcctcagtggaagtcggccagccgcctccgtgggagagaggcaggaaatcggaccaattcagtagcagtggggcttaaggtttatgaacggggtcttgagcggaggcctgagcgtacaaacagcttccccaccctcagcctcccggcgccatttcccttcactgggggtgggggatggggagctttcacatggcggacgctgccccgctggggtgaaagtggggcgcggaggcgggacttcttattccctttctaaagcacgctgcttcgggggccacggcgtctcctcggaaagctt

SEQ ID NO: 18 - DNA, 724 bp, Artificial Sequence
  Antibody (TRLH) light chain gene cDNA with optimized Kozak sequence added upstream of the initiation codon
cgcgccccgccgccaccatgggttggtcttgtatcatcttatttttagttgctactgctactggtgttcattctgatatacagatgacccaaagcccatcatctctgtctgcaagcgtcggcgacagggtgaccattacctgtcgcgcaagccaagacgttaatacagcagtggcttggtaccagcagaagcccggcaaggctcctaagctgctgatctatagcgcctcctttctttattctggagtgccttctcgtttttccggctcaaggtccggaactgattttaccctgaccatttcctccctccagcccgaggattttgccacttactactgtcagcagcactataccacaccacctacattcggacaaggtacaaaggtagaaatcaagcgtacggtggctgccccatccgtgttcatatttcctcctagcgacgaacaactcaagtccggtaccgccagcgtggtctgcctgttgaacaatttttatccaagagaagctaaggtccagtggaaggttgacaacgcccttcagtccggaaatagccaagagagcgtcaccgaacaggactccaaggacagtacatactcactgagctctacactgaccctttctaaggccgactacgagaagcacaaggtctacgcatgcgaagtgacccatcagggactcagtagccctgtaacaaagagttttaatcgaggcgagtgctaagcgat

SEQ ID NO: 19 - DNA, 1430 bp, Artificial Sequence
  Antibody (TRLH) heavy chain gene cDNA with optimized Kozak sequence added upstream of the initiation codon
ggccgcccgccgccaccatggaatttggtttatcttgggtttttttagttgctttattaagaggtgttcaatgtgaggtgcagttggtcgaatccggcggcggactcgtgcaaccaggcggaagtttgcggctgtcctgcgcagcctctggttttaacatcaaagatacctatattcattgggtacgccaggctcctggaaaggggcttgagtgggtggctcgaatttacccaaccaatggctacactcggtatgccgacagcgtcaaaggcagattcaccatctctgcagacacatcaaagaataccgcttacctgcagatgaactcactgagggccgaagataccgcagtttactactgctccaggtgggggggggacggcttctacgccatggattactggggacagggcacactcgtgaccgttagtagcgctagcaccaaaggcccctctgtgttcccacttgctccctccagtaaatctacctccggaggaaccgcagccctcggctgcctggtgaaggattacttcccagagcccgtcaccgtctcttggaactccggagccttgactagcggagtgcacactttccctgctgtattgcagtccagcggcttgtattcactgagtagcgtcgtcaccgtgccttcaagcagcctcgggacacagacatacatatgtaatgtcaaccataagccatcaaacactaaagttgataaaaaggtggaacctaagagttgcgataagacccatacctgtcctccttgccctgctcctgagctgctgggaggccctagcgtgtttctgttcccccccaagcccaaagatacactgatgatttcccgcacacctgaagtaacatgtgtcgtggttgatgtgagtcacgaggatccagaggtcaagtttaattggtacgtggacggagtggaggtgcacaacgctaagactaagcctcgggaggaacagtacaacagcacataccgcgtggtcagcgttttgactgtgctgcatcaagactggctcaatggaaaggaatacaagtgcaaggtctctaataaagccctccccgctcctattgagaagactatttctaaagccaagggccagcctcgcgaacctcaggtatatactttgccaccctctcgcgaagaaatgacaaagaatcaggtctcactcacttgcctcgtcaaagggttttacccttctgacatcgctgtcgaatgggaaagtaatggtcagccagaaaacaattacaagactactccaccagtgctcgattctgatggaagtttctttctctacagtaagctcactgtggacaaatctcgctggcagcagggtaacgtattctcatgctccgtgatgcatgaagccctccacaaccattacacccagaagagcctgtctctgagcccaggctaacctgca